European Patent Specification EP 3 280 445 B1, published January 17, 2024. Title: GENE THERAPY TO PREVENT REACTIONS TO ALLERGENS. Applicant: Cornell University. The sequence listing filed with the application follows.

SEQUENCE LISTING (11 sequences)

SEQ ID NO: 1 - DNA, 36 bp, Artificial Sequence
  Synthetic Heavy Chain CDR-H3
cgccgtgagcggctacagcatcaccagcggctacag

SEQ ID NO: 2 - DNA, 30 bp, Artificial Sequence
  Synthetic Heavy Chain CDR-H2
cagcatcacctacgacggcagcaccaacta

SEQ ID NO: 3 - DNA, 42 bp, Artificial Sequence
  Synthetic Heavy Chain CDR-H3
cgctcggggcagccactacttcggccactggcacttcgccgt

SEQ ID NO: 4 - DNA, 45 bp, Artificial Sequence
  Synthetic Light Chain CDR-L1
ccgggctagccagagcgtggactacgacggcgacagctacatgaa

SEQ ID NO: 5 - DNA, 24 bp, Artificial Sequence
  Synthetic Light Chain CDR-L2
ctacgctgccagctacctggagag

SEQ ID NO: 6 - DNA, 27 bp, Artificial Sequence
  Synthetic Light Chain CDR-L3
ccagcagagccacgaggacccctacac

SEQ ID NO: 7 - DNA, 363 bp, Artificial Sequence
  Synthetic Heavy Chain Variable Region
gaggtgcagctggtggagagcggcggtggcctggtgcagcctggtggtagcctgcgcctgagctgcgccgtgagcggctacagcatcaccagcggctacagctggaactggatccggcaggcccctggcaagggcctggagtgggtggccagcatcacctacgacggcagcaccaactacgccgacagcgtgaagggccggttcaccatcagccgggacgacagcaagaacaccttctacctgcagatgaactccctgcgggccgaggacaccgccgtgtactactgcgctcggggcagccactacttcggccactggcacttcgccgtgtggggtcagggcaccctggtgaccgtgagcagc

SEQ ID NO: 8 - DNA, 330 bp, Artificial Sequence
  Synthetic Light Chain Variable Region
gacatccagctgacccagagccctagcagcctgagcgccagcgtgggcgaccgggtgaccatcacctgccgggctagccagagcgtggactacgacggcgacagctacatgaattggtaccagcagaagcccggcaaggctcccaagctgctgatctacgctgccagctacctggagagcggcgtgcccagccggttcagcggcagcggcagcggcaccgacttcaccctgaccatcagcagcctgcagcccgaggacttcgccacctactactgccagcagagccacgaggacccctacaccttcggccagggcaccaaggtggagatc

SEQ ID NO: 9 - DNA, 2214 bp, Artificial Sequence
  Synthetic Anti-IgE antibody
atggagttcggcctgagctggctgttcctggtggccatcctgaagggcgtgcagtgcgaggtgcagctggtggagagcggcggtggcctggtgcagcctggtggtagcctgcgcctgagctgcgccgtgagcggctacagcatcaccagcggctacagctggaactggatccggcaggcccctggcaagggcctggagtgggtggccagcatcacctacgacggcagcaccaactacgccgacagcgtgaagggccggttcaccatcagccgggacgacagcaagaacaccttctacctgcagatgaactccctgcgggccgaggacaccgccgtgtactactgcgctcggggcagccactacttcggccactggcacttcgccgtgtggggtcagggcaccctggtgaccgtgagcagcgccagcaccaagggccccagcgtgttccctctggctccctcttccaaatccaccagcggcggcaccgctgccctgggctgcctggtgaaggactacttccccgagcccgtgaccgtgagctggaacagcggcgccctgaccagcggcgtgcacaccttccctgccgtgctgcaatccagcggcctgtacagcctgagcagcgtcgtgaccgtgcccagcagcagcctgggcacccagacctacatctgcaacgtgaaccacaagcccagcaacaccaaggtggacaagaaggccgagcccaagagctgcgacaagacccacacctgccctccctgccccgcccctgagctgctcggcggacccagcgtgttcctgttccctcccaagcccaaggacaccctgatgatcagccggacccctgaggtgacctgcgtggtcgtggacgtgagccacgaggaccccgaggtgaagttcaactggtatgtggacggcgtggaggtgcacaacgccaagaccaagccccgggaggagcagtacaacagcacctaccgggtggtgagcgtgctgaccgtgctgcaccaggactggctgaacggcaaggagtacaagtgcaaggtctccaacaaggccctgcctgcccctatcgagaagaccatcagcaaggccaagggccagccccgggagccccaggtgtacaccctgcctcctagccgggacgagctgaccaagaaccaggtctccctgacctgcctggtgaagggcttctaccccagcgacatcgccgtggagtgggagagcaacggccagcccgagaacaactacaagaccacccctcccgtgctggacagcgacggcagcttcttcctgtactccaagctgaccgtggacaagagccggtggcagcagggcaacgtgttcagctgcagcgtgatgcacgaggccctgcacaaccactacacccagaagagcctgagcctgagccccggacggaagcggaggagcggcgctcctgtgaagcagaccctgaacttcgacctgctgaagctggccggcgacgtggagagcaaccctgggcctatgaagtacctgctgcccaccgccgctgctggcctgctcctgctcgctgcccaacccgctgctgacatccagctgacccagagccctagcagcctgagcgccagcgtgggcgaccgggtgaccatcacctgccgggctagccagagcgtggactacgacggcgacagctacatgaattggtaccagcagaagcccggcaaggctcccaagctgctgatctacgctgccagctacctggagagcggcgtgcccagccggttcagcggcagcggcagcggcaccgacttcaccctgaccatcagcagcctgcagcccgaggacttcgccacctactactgccagcagagccacgaggacccctacaccttcggccagggcaccaaggtggagatcaagcggaccgtggccgctcctagcgtgttcatcttccctccctccgacgagcagctgaagagcggcaccgccagcgtggtgtgcctgctgaacaacttctaccctcgggaggccaaggtgcagtggaaggtggacaacgccctgcagagcggcaacagccaggagagcgtgaccgagcaggacagcaaggacagcacctacagcctgagcagcaccctgaccctgagcaaggccgactacgagaagcacaaggtgtacgcctgcgaggtgacccaccagggcctgagcagccccgtgaccaagagcttcaaccggggcgagtgc

SEQ ID NO: 10 - DNA, 1407 bp, Artificial Sequence
  Synthetic omalizumab heavy chain
atggagttcggcctgagctggctgttcctggtggccatcctgaagggcgtgcagtgcgaggtgcagctggtggagagcggcggtggcctggtgcagcctggtggtagcctgcgcctgagctgcgccgtgagcggctacagcatcaccagcggctacagctggaactggatccggcaggcccctggcaagggcctggagtgggtggccagcatcacctacgacggcagcaccaactacgccgacagcgtgaagggccggttcaccatcagccgggacgacagcaagaacaccttctacctgcagatgaactccctgcgggccgaggacaccgccgtgtactactgcgctcggggcagccactacttcggccactggcacttcgccgtgtggggtcagggcaccctggtgaccgtgagcagcgccagcaccaagggccccagcgtgttccctctggctccctcttccaaatccaccagcggcggcaccgctgccctgggctgcctggtgaaggactacttccccgagcccgtgaccgtgagctggaacagcggcgccctgaccagcggcgtgcacaccttccctgccgtgctgcaatccagcggcctgtacagcctgagcagcgtcgtgaccgtgcccagcagcagcctgggcacccagacctacatctgcaacgtgaaccacaagcccagcaacaccaaggtggacaagaaggccgagcccaagagctgcgacaagacccacacctgccctccctgccccgcccctgagctgctcggcggacccagcgtgttcctgttccctcccaagcccaaggacaccctgatgatcagccggacccctgaggtgacctgcgtggtcgtggacgtgagccacgaggaccccgaggtgaagttcaactggtatgtggacggcgtggaggtgcacaacgccaagaccaagccccgggaggagcagtacaacagcacctaccgggtggtgagcgtgctgaccgtgctgcaccaggactggctgaacggcaaggagtacaagtgcaaggtctccaacaaggccctgcctgcccctatcgagaagaccatcagcaaggccaagggccagccccgggagccccaggtgtacaccctgcctcctagccgggacgagctgaccaagaaccaggtctccctgacctgcctggtgaagggcttctaccccagcgacatcgccgtggagtgggagagcaacggccagcccgagaacaactacaagaccacccctcccgtgctggacagcgacggcagcttcttcctgtactccaagctgaccgtggacaagagccggtggcagcagggcaacgtgttcagctgcagcgtgatgcacgaggccctgcacaaccactacacccagaagagcctgagcctgagccccgga

SEQ ID NO: 11 - DNA, 645 bp, Artificial Sequence
  Synthetic omalizumab light chain
gacatccagctgacccagagccctagcagcctgagcgccagcgtgggcgaccgggtgaccatcacctgccgggctagccagagcgtggactacgacggcgacagctacatgaattggtaccagcagaagcccggcaaggctcccaagctgctgatctacgctgccagctacctggagagcggcgtgcccagccggttcagcggcagcggcagcggcaccgacttcaccctgaccatcagcagcctgcagcccgaggacttcgccacctactactgccagcagagccacgaggacccctacaccttcggccagggcaccaaggtggagatcaagcggaccgtggccgctcctagcgtgttcatcttccctccctccgacgagcagctgaagagcggcaccgccagcgtggtgtgcctgctgaacaacttctaccctcgggaggccaaggtgcagtggaaggtggacaacgccctgcagagcggcaacagccaggagagcgtgaccgagcaggacagcaaggacagcacctacagcctgagcagcaccctgaccctgagcaaggccgactacgagaagcacaaggtgtacgcctgcgaggtgacccaccagggcctgagcagccccgtgaccaagagcttcaaccgg